European Patent Application EP 4 177 345 A1, published May 10, 2023. Title: Improved RNA Editing Method. Applicant: EdiGene Inc. The sequence listing filed with the application follows.

SEQUENCE LISTING (76 sequences)

SEQ ID NO: 1 - DNA, 41 bp, Artificial Sequence
  PCR primer
ggagtgagtacggtgtgcgacgagctgtacaagctgcaggg

SEQ ID NO: 2 - DNA, 43 bp, Artificial Sequence
  PCR primer
gagttggatgctggatggtggtgcagatgaacttcagggtcag

SEQ ID NO: 3 - DNA, 56 bp, Artificial Sequence
  Vector-F
ctgttttgacctccatagaagacaccgactctagacgtggaacagtacgaacgcgc

SEQ ID NO: 4 - DNA, 36 bp, Artificial Sequence
  GAT-R
cactggcagagccctatcgcatcgcgagcaggcgct

SEQ ID NO: 5 - DNA, 33 bp, Artificial Sequence
  GAT-F
tgctcgcgatgcgatagggctctgccagtgagc

SEQ ID NO: 6 - DNA, 59 bp, Artificial Sequence
  Vector-R
gggtttaaacccctgcagggtgtacaccggcgcgccttacttgtacagctcgtccatgc

SEQ ID NO: 7 - DNA, 36 bp, Artificial Sequence
  GAA-R
cactggcagagccctttcgcatcgcgagcaggcgct

SEQ ID NO: 8 - DNA, 33 bp, Artificial Sequence
  GAA-F
tgctcgcgatgcgaaagggctctgccagtgagc

SEQ ID NO: 9 - DNA, 36 bp, Artificial Sequence
  GAG-R
cactggcagagccctctcgcatcgcgagcaggcgct

SEQ ID NO: 10 - DNA, 33 bp, Artificial Sequence
  GAG-F
tgctcgcgatgcgagagggctctgccagtgagc

SEQ ID NO: 11 - DNA, 36 bp, Artificial Sequence
  GAC-R
cactggcagagccctgtcgcatcgcgagcaggcgct

SEQ ID NO: 12 - DNA, 33 bp, Artificial Sequence
  GAC-F
tgctcgcgatgcgacagggctctgccagtgagc

SEQ ID NO: 13 - DNA, 36 bp, Artificial Sequence
  AAA-R
cactggcagagcccttttgcatcgcgagcaggcgct

SEQ ID NO: 14 - DNA, 33 bp, Artificial Sequence
  AAA-F
tgctcgcgatgcaaaagggctctgccagtgagc

SEQ ID NO: 15 - DNA, 36 bp, Artificial Sequence
  AAT-R
cactggcagagccctattgcatcgcgagcaggcgct

SEQ ID NO: 16 - DNA, 33 bp, Artificial Sequence
  AAT-F
tgctcgcgatgcaatagggctctgccagtgagc

SEQ ID NO: 17 - DNA, 36 bp, Artificial Sequence
  AAC-R
cactggcagagccctgttgcatcgcgagcaggcgct

SEQ ID NO: 18 - DNA, 33 bp, Artificial Sequence
  AAC-F
tgctcgcgatgcaacagggctctgccagtgagc

SEQ ID NO: 19 - DNA, 36 bp, Artificial Sequence
  AAG-R
cactggcagagccctcttgcatcgcgagcaggcgct

SEQ ID NO: 20 - DNA, 33 bp, Artificial Sequence
  AAG-F
tgctcgcgatgcaagagggctctgccagtgagc

SEQ ID NO: 21 - DNA, 36 bp, Artificial Sequence
  CAA-R
cactggcagagccctttggcatcgcgagcaggcgct

SEQ ID NO: 22 - DNA, 33 bp, Artificial Sequence
  CAA-F
tgctcgcgatgccaaagggctctgccagtgagc

SEQ ID NO: 23 - DNA, 36 bp, Artificial Sequence
  CAT-R
cactggcagagccctatggcatcgcgagcaggcgct

SEQ ID NO: 24 - DNA, 33 bp, Artificial Sequence
  CAT-F
tgctcgcgatgccatagggctctgccagtgagc

SEQ ID NO: 25 - DNA, 36 bp, Artificial Sequence
  CAC-R
cactggcagagccctgtggcatcgcgagcaggcgct

SEQ ID NO: 26 - DNA, 33 bp, Artificial Sequence
  CAC-F
tgctcgcgatgccacagggctctgccagtgagc

SEQ ID NO: 27 - DNA, 36 bp, Artificial Sequence
  CAG-R
cactggcagagccctctggcatcgcgagcaggcgct

SEQ ID NO: 28 - DNA, 33 bp, Artificial Sequence
  CAG-F
tgctcgcgatgccagagggctctgccagtgagc

SEQ ID NO: 29 - DNA, 36 bp, Artificial Sequence
  TAA-R
cactggcagagccctttagcatcgcgagcaggcgct

SEQ ID NO: 30 - DNA, 33 bp, Artificial Sequence
  TAA-F
tgctcgcgatgctaaagggctctgccagtgagc

SEQ ID NO: 31 - DNA, 36 bp, Artificial Sequence
  TAG-R
cactggcagagccctctagcatcgcgagcaggcgct

SEQ ID NO: 32 - DNA, 33 bp, Artificial Sequence
  TAG-F
tgctcgcgatgctagagggctctgccagtgagc

SEQ ID NO: 33 - DNA, 36 bp, Artificial Sequence
  TAC-R
cactggcagagccctgtagcatcgcgagcaggcgct

SEQ ID NO: 34 - DNA, 33 bp, Artificial Sequence
  TAC-F
tgctcgcgatgctacagggctctgccagtgagc

SEQ ID NO: 35 - DNA, 36 bp, Artificial Sequence
  TAT-R
cactggcagagccctatagcatcgcgagcaggcgct

SEQ ID NO: 36 - DNA, 33 bp, Artificial Sequence
  TAT-F
tgctcgcgatgctatagggctctgccagtgagc

SEQ ID NO: 37 - RNA, 81 nt, Artificial Sequence
  arRNA-UCU
gaugggcaccaccccggugaacagcuccucgcccuugcucacuggcagagcccuucugcaucgcgagcaggcgcugccucc

SEQ ID NO: 38 - RNA, 81 nt, Artificial Sequence
  arRNA-ACU
gaugggcaccaccccggugaacagcuccucgcccuugcucacuggcagagcccuacugcaucgcgagcaggcgcugccucc

SEQ ID NO: 39 - RNA, 81 nt, Artificial Sequence
  arRNA-GCU
gaugggcaccaccccggugaacagcuccucgcccuugcucacuggcagagcccugcugcaucgcgagcaggcgcugccucc

SEQ ID NO: 40 - RNA, 81 nt, Artificial Sequence
  arRNA-CCU
gaugggcaccaccccggugaacagcuccucgcccuugcucacuggcagagcccuccugcaucgcgagcaggcgcugccucc

SEQ ID NO: 41 - RNA, 81 nt, Artificial Sequence
  arRNA-UCA
gaugggcaccaccccggugaacagcuccucgcccuugcucacuggcagagcccuucagcaucgcgagcaggcgcugccucc

SEQ ID NO: 42 - RNA, 81 nt, Artificial Sequence
  arRNA-ACA
gaugggcaccaccccggugaacagcuccucgcccuugcucacuggcagagcccuacagcaucgcgagcaggcgcugccucc

SEQ ID NO: 43 - RNA, 81 nt, Artificial Sequence
  arRNA-GCA
gaugggcaccaccccggugaacagcuccucgcccuugcucacuggcagagcccugcagcaucgcgagcaggcgcugccucc

SEQ ID NO: 44 - RNA, 81 nt, Artificial Sequence
  arRNA-CCA
gaugggcaccaccccggugaacagcuccucgcccuugcucacuggcagagcccuccagcaucgcgagcaggcgcugccucc

SEQ ID NO: 45 - RNA, 81 nt, Artificial Sequence
  arRNA-UCG
gaugggcaccaccccggugaacagcuccucgcccuugcucacuggcagagcccuucggcaucgcgagcaggcgcugccucc

SEQ ID NO: 46 - RNA, 81 nt, Artificial Sequence
  arRNA-ACG
gaugggcaccaccccggugaacagcuccucgcccuugcucacuggcagagcccuacggcaucgcgagcaggcgcugccucc

SEQ ID NO: 47 - RNA, 81 nt, Artificial Sequence
  arRNA-GCG
gaugggcaccaccccggugaacagcuccucgcccuugcucacuggcagagcccugcggcaucgcgagcaggcgcugccucc

SEQ ID NO: 48 - RNA, 81 nt, Artificial Sequence
  arRNA-CCG
gaugggcaccaccccggugaacagcuccucgcccuugcucacuggcagagcccuccggcaucgcgagcaggcgcugccucc

SEQ ID NO: 49 - RNA, 81 nt, Artificial Sequence
  arRNA-UCC
gaugggcaccaccccggugaacagcuccucgcccuugcucacuggcagagcccuuccgcaucgcgagcaggcgcugccucc

SEQ ID NO: 50 - RNA, 81 nt, Artificial Sequence
  arRNA-ACC
gaugggcaccaccccggugaacagcuccucgcccuugcucacuggcagagcccuaccgcaucgcgagcaggcgcugccucc

SEQ ID NO: 51 - RNA, 81 nt, Artificial Sequence
  arRNA-GCC
gaugggcaccaccccggugaacagcuccucgcccuugcucacuggcagagcccugccgcaucgcgagcaggcgcugccucc

SEQ ID NO: 52 - RNA, 81 nt, Artificial Sequence
  arRNA-CCC
gaugggcaccaccccggugaacagcuccucgcccuugcucacuggcagagcccucccgcaucgcgagcaggcgcugccucc

SEQ ID NO: 53 - RNA, 91 nt, Artificial Sequence
  arRNA-random
caauaggcacuaacuuauuggcgcuggugaacggacuuccucucgaguaccagaagaugacuacaaaacuccuuuccauugcgaguaucgg

SEQ ID NO: 54 - DNA, 9088 bp, Artificial Sequence
  Reference sequence of Reporter 1
ctaggcttttgcaaaaagctatcgctagctcgagcacgtgttgacaattaatcatcggcatagtatatcggcatagtataatacgacaaggtgaggaactaaaccatggccaagcctttgtctcaagaagaatccaccctcattgaaagagcaacggctacaatcaacagcatccccatctctgaagactacagcgtcgccagcgcagctctctctagcgacggccgcatcttcactggtgtcaatgtatatcattttactgggggaccttgtgcagaactcgtggtgctgggcactgctgctgctgcggcagctggcaacctgacttgtatcgtcgcgatcggaaatgagaacaggggcatcttgagcccctgcggacggtgccgacaggtgcttctcgatctgcatcctgggatcaaagccatagtgaaggacagtgatggacagccgacggcagttgggattcgtgaattgctgccctctggttatgtgtgggagggctaagcacttcgtggccgaggagcaggactgagaattccagtcgacaatcaacctctggattacaaaatttgtgaaagattgactggtattcttaactatgttgctccttttacgctatgtggatacgctgctttaatgcctttgtatcatgctattgcttcccgtatggctttcattttctcctccttgtataaatcctggttgctgtctctttatgaggagttgtggcccgttgtcaggcaacgtggcgtggtgtgcactgtgtttgctgacgcaacccccactggttggggcattgccaccacctgtcagctcctttccgggactttcgctttccccctccctattgccacggcggaactcatcgccgcctgccttgcccgctgctggacaggggctcggctgttgggcactgacaattccgtggtgttgtcggggaagctgacgtcctttccatggctgctcgcctgtgttgccacctggattctgcgcgggacgtccttctgctacgtcccttcggccctcaatccagcggaccttccttcccgcggcctgctgccggctctgcggcctcttccgcgtcttcgccttcgccctcagacgagtcggatctccctttgggccgcctccccgcctggaattcgagctcggtacctttaagaccaatgacttacaaggcagctgtagatcttagccactttttaaaagaaaaggggggactggaagggctaattcactcccaacgaagacaagatctgctttttgcttgtactgggtctctctggttagaccagatctgagcctgggagctctctggctaactagggaacccactgcttaagcctcaataaagcttgccttgagtgcttcaagtagtgtgtgcccgtctgttgtgtgactctggtaactagagatccctcagacccttttagtcagtgtggaaaatctctagcagtagtagttcatgtcatcttattattcagtatttataacttgcaaagaaatgaatatcagagagtgagaggaacttgtttattgcagcttataatggttacaaataaagcaatagcatcacaaatttcacaaataaagcatttttttcactgcattctagttgtggtttgtccaaactcatcaatgtatcttatcatgtctggctctagctatcccgcccctaactccgcccagttccgcccattctccgccccatggctgactaattttttttatttatgcagaggccgaggccgcctcggcctctgagctattccagaagtagtgaggaggcttttttggaggcctaggcttttgcgtcgagacgtacccaattcgccctatagtgagtcgtattacgcgcgctcactggccgtcgttttacaacgtcgtgactgggaaaaccctggcgttacccaacttaatcgccttgcagcacatccccctttcgccagctggcgtaatagcgaagaggcccgcaccgatcgcccttcccaacagttgcgcagcctgaatggcgaatggcgcgacgcgccctgtagcggcgcattaagcgcggcgggtgtggtggttacgcgcagcgtgaccgctacacttgccagcgccctagcgcccgctcctttcgctttcttcccttcctttctcgccacgttcgccggctttccccgtcaagctctaaatcgggggctccctttagggttccgatttagtgctttacggcacctcgaccccaaaaaacttgattagggtgatggttcacgtagtgggccatcgccctgatagacggtttttcgccctttgacgttggagtccacgttctttaatagtggactcttgttccaaactggaacaacactcaaccctatctcggtctattcttttgatttataagggattttgccgatttcggcctattggttaaaaaatgagctgatttaacaaaaatttaacgcgaattttaacaaaatattaacgtttacaatttcccaggtggcacttttcggggaaatgtgcgcggaacccctatttgtttatttttctaaatacattcaaatatgtatccgctcatgagacaataaccctgataaatgcttcaataatattgaaaaaggaagagtatgagtattcaacatttccgtgtcgcccttattcccttttttgcggcattttgccttcctgtttttgctcacccagaaacgctggtgaaagtaaaagatgctgaagatcagttgggtgcacgagtgggttacatcgaactggatctcaacagcggtaagatccttgagagttttcgccccgaagaacgttttccaatgatgagcacttttaaagttctgctatgtggcgcggtattatcccgtattgacgccgggcaagagcaactcggtcgccgcatacactattctcagaatgacttggttgagtactcaccagtcacagaaaagcatcttacggatggcatgacagtaagagaattatgcagtgctgccataaccatgagtgataacactgcggccaacttacttctgacaacgatcggaggaccgaaggagctaaccgcttttttgcacaacatgggggatcatgtaactcgccttgatcgttgggaaccggagctgaatgaagccataccaaacgacgagcgtgacaccacgatgcctgtagcaatggcaacaacgttgcgcaaactattaactggcgaactacttactctagcttcccggcaacaattaatagactggatggaggcggataaagttgcaggaccacttctgcgctcggcccttccggctggctggtttattgctgataaatctggagccggtgagcgtgggtctcgcggtatcattgcagcactggggccagatggtaagccctcccgtatcgtagttatctacacgacggggagtcaggcaactatggatgaacgaaatagacagatcgctgagataggtgcctcactgattaagcattggtaactgtcagaccaagtttactcatatatactttagattgatttaaaacttcatttttaatttaaaaggatctaggtgaagatcctttttgataatctcatgaccaaaatcccttaacgtgagttttcgttccactgagcgtcagaccccgtagaaaagatcaaaggatcttcttgagatcctttttttctgcgcgtaatctgctgcttgcaaacaaaaaaaccaccgctaccagcggtggtttgtttgccggatcaagagctaccaactctttttccgaaggtaactggcttcagcagagcgcagataccaaatactgtccttctagtgtagccgtagttaggccaccacttcaagaactctgtagcaccgcctacatacctcgctctgctaatcctgttaccagtggctgctgccagtggcgataagtcgtgtcttaccgggttggactcaagacgatagttaccggataaggcgcagcggtcgggctgaacggggggttcgtgcacacagcccagcttggagcgaacgacctacaccgaactgagatacctacagcgtgagctatgagaaagcgccacgcttcccgaagggagaaaggcggacaggtatccggtaagcggcagggtcggaacaggagagcgcacgagggagcttccagggggaaacgcctggtatctttatagtcctgtcgggtttcgccacctctgacttgagcgtcgatttttgtgatgctcgtcaggggggcggagcctatggaaaaacgccagcaacgcggcctttttacggttcctggccttttgctggccttttgctcacatgttctttcctgcgttatcccctgattctgtggataaccgtattaccgcctttgagtgagctgataccgctcgccgcagccgaacgaccgagcgcagcgagtcagtgagcgaggaagcggaagagcgcccaatacgcaaaccgcctctccccgcgcgttggccgattcattaatgcagctggcacgacaggtttcccgactggaaagcgggcagtgagcgcaacgcaattaatgtgagttagctcactcattaggcaccccaggctttacactttatgcttccggctcgtatgttgtgtggaattgtgagcggataacaatttcacacaggaaacagctatgaccatgattacgccaagcgcgcaattaaccctcactaaagggaacaaaagctggagctgcaagcttaatgtagtcttatgcaatactcttgtagtcttgcaacatggtaacgatgagttagcaacatgccttacaaggagagaaaaagcaccgtgcatgccgattggtggaagtaaggtggtacgatcgtgccttattaggaaggcaacagacgggtctgacatggattggacgaaccactgaattgccgcattgcagagatattgtatttaagtgcctagctcgatacaataaacgggtctctctggttagaccagatctgagcctgggagctctctggctaactagggaacccactgcttaagcctcaataaagcttgccttgagtgcttcaagtagtgtgtgcccgtctgttgtgtgactctggtaactagagatccctcagacccttttagtcagtgtggaaaatctctagcagtggcgcccgaacagggacctgaaagcgaaagggaaaccagagctctctcgacgcaggactcggcttgctgaagcgcgcacggcaagaggcgaggggcggcgactggtgagtacgccaaaaattttgactagcggaggctagaaggagagagatgggtgcgagagcgtcagtattaagcgggggagaattagatcgcgatgggaaaaaattcggttaaggccagggggaaagaaaaaatataaattaaaacatatagtatgggcaagcagggagctagaacgattcgcagttaatcctggcctgttagaaacatcagaaggctgtagacaaatactgggacagctacaaccatcccttcagacaggatcagaagaacttagatcattatataatacagtagcaaccctctattgtgtgcatcaaaggatagagataaaagacaccaaggaagctttagacaagatagaggaagagcaaaacaaaagtaagaccaccgcacagcaagcggccgctgatcttcagacctggaggaggagatatgagggacaattggagaagtgaattatataaatataaagtagtaaaaattgaaccattaggagtagcacccaccaaggcaaagagaagagtggtgcagagagaaaaaagagcagtgggaataggagctttgttccttgggttcttgggagcagcaggaagcactatgggcgcagcctcaatgacgctgacggtacaggccagacaattattgtctggtatagtgcagcagcagaacaatttgctgagggctattgaggcgcaacagcatctgttgcaactcacagtctggggcatcaagcagctccaggcaagaatcctggctgtggaaagatacctaaaggatcaacagctcctggggatttggggttgctctggaaaactcatttgcaccactgctgtgccttggaatgctagttggagtaataaatctctggaacagattggaatcacacgacctggatggagtgggacagagaaattaacaattacacaagcttaatacactccttaattgaagaatcgcaaaaccagcaagaaaagaatgaacaagaattattggaattagataaatgggcaagtttgtggaattggtttaacataacaaattggctgtggtatataaaattattcataatgatagtaggaggcttggtaggtttaagaatagtttttgctgtactttctatagtgaatagagttaggcagggatattcaccattatcgtttcagacccacctcccaaccccgaggggacccgacaggcccgaaggaatagaagaagaaggtggagagagagacagagacagatccattcgattagtgaacggatctcgacggttaacttttaaaagaaaaggggggattggggggtacagtgcaggggaaagaatagtagacataatagcaacagacatacaaactaaagaattacaaaaacaaattacaaaaattcaaaattttatcgataagcttgggagttccgcgttacataacttacggtaaatggcccgcctggctgaccgcccaacgacccccgcccattgacgtcaataatgacgtatgttcccatagtaacgccaatagggactttccattgacgtcaatgggtggagtatttacggtaaactgcccacttggcagtacatcaagtgtatcatatgccaagtacgccccctattgacgtcaatgacggtaaatggcccgcctggcattatgcccagtacatgaccttatgggactttcctacttggcagtacatctacgtattagtcatcgctattaccatggtgatgcggttttggcagtacatcaatgggcgtggatagcggtttgactcacggggatttccaagtctccaccccattgacgtcaatgggagtttgttttggcaccaaaatcaacgggactttccaaaatgtcgtaacaactccgccccattgacgcaaatgggcggtaggcgtgtacggtgggaggtctatataagcagagctcgtttagtgaaccgtcagatcgcctggagacgccatccacgctgttttgacctccatagaagacaccgactctagaggatccggactagtatggtgagcaagggcgaggaggataacatggccatcatcaaggagttcatgcgcttcaaggtgcacatggagggctccgtgaacggccacgagttcgagatcgagggcgagggcgagggccgcccctacgagggcacccagaccgccaagctgaaggtgaccaagggtggccccctgcccttcgcctgggacatcctgtcccctcagttcatgtacggctccaaggcctacgtgaagcaccccgccgacatccccgactacttgaagctgtccttccccgagggcttcaagtgggagcgcgtgatgaacttcgaggacggcggcgtggtgaccgtgacccaggactcctccctgcaggacggcgagttcatctacaaggtgaagctgcgcggcaccaacttcccctccgacggccccgtaatgcagaagaagaccatgggctgggaggcctcctccgagcggatgtaccccgaggacggcgccctgaagggcgagatcaagcagaggctgaagctgaaggacggcggccactacgacgctgaggtcaagaccacctacaaggccaagaagcccgtgcagctgcccggcgcctacaacgtcaacatcaagttggacatcacctcccacaacgaggactacaccatcgtggaacagtacgaacgcgccgagggccgccactccaccggcggcatggacgagctgtacaagctgcagggcggaggaggcagcgcctgctcgcgatgcgatagggctctgccagtgagcaagggcgaggagctgttcaccggggtggtgcccatcctggtcgagctggacggcgacgtaaacggccacaagttcagcgtgtccggcgagggcgagggcgatgccacctacggcaagctgaccctgaagttcatctgcaccaccggcaagctgcccgtgccctggcccaccctcgtgaccaccctgacctacggcgtgcagtgcttcagccgctaccccgaccacatgaagcagcacgacttcttcaagtccgccatgcccgaaggctacgtccaggagcgcaccatcttcttcaaggacgacggcaactacaagacccgcgccgaggtgaagttcgagggcgacaccctggtgaaccgcatcgagctgaagggcatcgacttcaaggaggacggcaacatcctggggcacaagctggagtacaactacaacagccacaacgtctatatcatggccgacaagcagaagaacggcatcaaggtgaacttcaagatccgccacaacatcgaggacggcagcgtgcagctcgccgaccactaccagcagaacacccccatcggcgacggccccgtgctgctgcccgacaaccactacctgagcacccagtccgccctgagcaaagaccccaacgagaagcgcgatcacatggtcctgctggagttcgtgaccgccgccgggatcactctcggcatggacgagctgtacaagtaaggcgcgccggtgtacaccctgcaggggtttaaacccacgcgtcgaccagtggtcgaccctgtggaatgtgtgtcagttagggtgtggaaagtccccaggctccccagcaggcagaagtatgcaaagcatgcatctcaattagtcagcaaccaggtgtggaaagtccccaggctccccagcaggcagaagtatgcaaagcatgcatctcaattagtcagcaaccatagtcccgcccctaactccgcccatcccgcccctaactccgcccagttccgcccattctccgccccatggctgactaattttttttatttatgcagaggccgaggccgcctcggcctctgagctattccagaagtagtgaggaggcttttttggaggc

SEQ ID NO: 55 - RNA, 91 nt, Artificial Sequence
  arRNA-UAG
gcugcuucauguggucgggguagcggcugaagcacugcacgccguaggucaggguggucacgagggugggccagggcacgggcagcuugcc

SEQ ID NO: 56 - RNA, 91 nt, Artificial Sequence
  arRNA-UUG
gcugcuucauguggucgggguagcggcugaagcacugcacgccguuggucaggguggucacgagggugggccagggcacgggcagcuugcc

SEQ ID NO: 57 - RNA, 91 nt, Artificial Sequence
  arRNA-UCG
gcugcuucauguggucgggguagcggcugaagcacugcacgccgucggucaggguggucacgagggugggccagggcacgggcagcuugcc

SEQ ID NO: 58 - RNA, 91 nt, Artificial Sequence
  arRNA-UGG
gcugcuucauguggucgggguagcggcugaagcacugcacgccgugggucaggguggucacgagggugggccagggcacgggcagcuugcc

SEQ ID NO: 59 - DNA, 2130 bp, Artificial Sequence
  Full-length cDNA sequence of ADAR2-r16
atggatatagaagatgaagaaaacatgagttccagcagcactgatgtgaaggaaaaccgcaatctggacaacgtgtcccccaaggatggcagcacacctgggcctggcgagggctctcagctctccaatgggggtggtggtggccccggcagaaagcggcccctggaggagggcagcaatggccactccaagtaccgcctgaagaaaaggaggaaaacaccagggcccgtcctccccaagaacgccctgatgcagctgaatgagatcaagcctggtttgcagtacacactcctgtcccagactgggcccgtgcacgcgcctttgtttgtcatgtctgtggaggtgaatggccaggtttttgagggctctggtcccacaaagaaaaaggcaaaactccatgctgctgagaaggccttgaggtctttcgttcagtttcctaatgcctctgaggcccacctggccatggggaggaccctgtctgtcaacacggacttcacatctgaccaggccgacttccctgacacgctcttcaatggttttgaaactcctgacaaggcggagcctcccttttacgtgggctccaatggggatgactccttcagttccagcggggacctcagcttgtctgcttccccggtgcctgccagcctagcccagcctcctctccctgccttaccaccattcccacccccgagtgggaagaatcccgtgatgatcttgaacgaactgcgcccaggactcaagtatgacttcctctccgagagcggggagagccatgccaagagcttcgtcatgtctgtggtcgtggatggtcagttctttgaaggctcggggagaaacaagaagcttgccaaggcccgggctgcgcagtctgccctggccgccatttttaacttgcacttggatcagacgccatctcgccagcctattcccagtgagggtcttcagctgcatttaccgcaggttttagctgacgctgtctcacgcctggtcataggtaagtttggtgacctgaccgacaacttctcctcccctcacgctcgcagaataggtctggctggagtcgtcatgacaacaggcacagatgttaaagatgccaaggtgatatgtgtttctacaggatctaaatgtattaatggtgaatacctaagtgatcgtggccttgcattaaatgactgccatgcagaaatagtatctcggagatccttgctcagatttctttatacacaacttgagctttacttaaataacgaggatgatcaaaaaagatccatctttcagaaatcagagcgaggggggtttaggctgaaggagaatatacagtttcatctgtacatcagcacctctccctgtggagatgccagaatcttctcaccacatgaggcaatcctggaagaaccagcagatagacacccaaatcgtaaagcaagaggacagctacggaccaaaatagaggctggtcaggggacgattccagtgcgcaacaatgcgagcatccaaacgtgggacggggtgctgcaaggggagcggctgctcaccatgtcctgcagtgacaagattgcacgctggaacgtggtgggcatccagggatcactgctcagcattttcgtggagcccatttacttctcgagcatcatcctgggcagcctttaccacggggaccacctttccagggccatgtaccagcggatctccaacatagaggacctgccacctctctacaccctcaacaagcctttgctcacaggcatcagcaatgcagaagcacggcagccagggaaggcccccatattcagtgtcaactggacggtaggcgactccgctattgaggtcatcaacgccacgactgggaagggagagctgggccgcgcgtcccgcctgtgtaagcacgcgttgtactgtcgctggatgcgtgtgcacggcaaggttccctcccacttactacgctccaagattaccaagcccaacgtgtaccatgagacaaagctggcggcaaaggagtaccaggccgccaaggcgcgtctgttcacagccttcatcaaggcggggctgggggcctgggtggagaagcccaccgagcaggaccagttctcactcacgcccgattacaaggatgacgacgataagtag

SEQ ID NO: 60 - DNA, 720 bp, Artificial Sequence
  BFP cDNA sequence
atggtgagcaagggcgaggagctgttcaccggggtggtgcccatcctggtcgagctggacggcgacgtaaacggccacaagttcagcgtgtctggcgagggcgagggcgatgccacctacggcaagctgaccctgaagttcatctgcaccaccggcaagctgcccgtgccctggcccaccctcgtgaccaccctgacccacggcgtgcagtgcttcagccgctaccccgaccacatgaagcagcacgacttcttcaagtccgccatgcccgaaggctacgtccaggagcgcaccatcttcttcaaggacgacggcaactacaagacccgcgccgaggtgaagttcgagggcgacaccctggtgaaccgcatcgagctgaagggcatcgacttcaaggaggacggcaacatcctggggcacaagctggagtacaactacaacagccacaacgtctatatcatggccgacaagcagaagaacggcatcaaggcgaacttcaagatccgccacaacatcgaggacggcagcgtgcagctcgccgaccactaccagcagaacacccccatcggcgacggccccgtgctgctgcccgacaaccactacctgagcacccagtccgccctgagcaaagaccccaacgagaagcgcgatcacatggtcctgctggagttcgtgaccgccgccgggatcactctcggcatggacgagctgtacaagtga

SEQ ID NO: 61 - RNA, 91 nt, Artificial Sequence
  arRNA-UUU
gcugcuucauguggucgggguagcggcugaagcacugcacgccguuugucaggguggucacgagggugggccagggcacgggcagcuugcc

SEQ ID NO: 62 - RNA, 91 nt, Artificial Sequence
  arRNA-AUU
gcugcuucauguggucgggguagcggcugaagcacugcacgccgauugucaggguggucacgagggugggccagggcacgggcagcuugcc

SEQ ID NO: 63 - RNA, 91 nt, Artificial Sequence
  arRNA-GUU
gcugcuucauguggucgggguagcggcugaagcacugcacgccgguugucaggguggucacgagggugggccagggcacgggcagcuugcc

SEQ ID NO: 64 - RNA, 91 nt, Artificial Sequence
  arRNA-CUU
gcugcuucauguggucgggguagcggcugaagcacugcacgccgcuugucaggguggucacgagggugggccagggcacgggcagcuugcc

SEQ ID NO: 65 - RNA, 91 nt, Artificial Sequence
  arRNA-UUA
gcugcuucauguggucgggguagcggcugaagcacugcacgccguuagucaggguggucacgagggugggccagggcacgggcagcuugcc

SEQ ID NO: 66 - RNA, 91 nt, Artificial Sequence
  arRNA-AUA
gcugcuucauguggucgggguagcggcugaagcacugcacgccgauagucaggguggucacgagggugggccagggcacgggcagcuugcc

SEQ ID NO: 67 - RNA, 91 nt, Artificial Sequence
  arRNA-GUA
gcugcuucauguggucgggguagcggcugaagcacugcacgccgguagucaggguggucacgagggugggccagggcacgggcagcuugcc

SEQ ID NO: 68 - RNA, 91 nt, Artificial Sequence
  arRNA-CUA
gcugcuucauguggucgggguagcggcugaagcacugcacgccgcuagucaggguggucacgagggugggccagggcacgggcagcuugcc

SEQ ID NO: 69 - RNA, 91 nt, Artificial Sequence
  arRNA-AUG
gcugcuucauguggucgggguagcggcugaagcacugcacgccgauggucaggguggucacgagggugggccagggcacgggcagcuugcc

SEQ ID NO: 70 - RNA, 91 nt, Artificial Sequence
  arRNA-GUG
gcugcuucauguggucgggguagcggcugaagcacugcacgccgguggucaggguggucacgagggugggccagggcacgggcagcuugcc

SEQ ID NO: 71 - RNA, 91 nt, Artificial Sequence
  arRNA-CUG
gcugcuucauguggucgggguagcggcugaagcacugcacgccgcuggucaggguggucacgagggugggccagggcacgggcagcuugcc

SEQ ID NO: 72 - RNA, 91 nt, Artificial Sequence
  arRNA-UUC
gcugcuucauguggucgggguagcggcugaagcacugcacgccguucgucaggguggucacgagggugggccagggcacgggcagcuugcc

SEQ ID NO: 73 - RNA, 91 nt, Artificial Sequence
  arRNA-AUC
gcugcuucauguggucgggguagcggcugaagcacugcacgccgaucgucaggguggucacgagggugggccagggcacgggcagcuugcc

SEQ ID NO: 74 - RNA, 91 nt, Artificial Sequence
  arRNA-GUC
gcugcuucauguggucgggguagcggcugaagcacugcacgccggucgucaggguggucacgagggugggccagggcacgggcagcuugcc

SEQ ID NO: 75 - RNA, 91 nt, Artificial Sequence
  arRNA-CUC
gcugcuucauguggucgggguagcggcugaagcacugcacgccgcucgucaggguggucacgagggugggccagggcacgggcagcuugcc

SEQ ID NO: 76 - RNA, 91 nt, Artificial Sequence
  Ran-91
uaauccugaauaucgcgcaauuccccagcagagaacaucgcggugugaacgucccuuuauaccgggcagguauagcugaaaucagcguggc